European Patent Specification EP 3 679 069 B1, published November 20, 2024. Title: Antibodies useful in cancer diagnosis. Applicant: Ganymed Pharmaceuticals GmbH et al. The sequence listing filed with the application follows.

SEQUENCE LISTING (61 sequences)

SEQ ID NO: 1 - protein, 220 aa, Homo sapiens
MASAGMQILGVVLTLLGWVNGLVSCALPMWKVTAFIGNSIVVAQVVWEGLWMSCVVQSTGQMQCKVYDSLLALPQDLQAARALCVIALLVALFGLLVYLAGAKCTTCVEEKDSKARLVLTSGIVFVISGVLTLIPVCWTAHAIIRDFYNPLVAEAQKRELGASLYLGWAASGLLLLGGGLLCCTCPSGGSQGPSHYMARYSTSAPAISRGPSEYPTKNYV

SEQ ID NO: 2 - protein, 217 aa, Homo sapiens
MASTGLELLGMTLAVLGWLGTLVSCALPLWKVTAFIGNSIVVAQVVWEGLWMSCVVQSTGQMQCKVYDSLLALPQDLQAARALCVIALLLALLGLLVAITGAQCTTCVEDEGAKARIVLTAGVILLLAGILVLIPVCWTAHAIIQDFYNPLVAEALKRELGASLYLGWAAAALLMLGGGLLCCTCPPPQVERPRGPRLGYSIPSRSGASGLDKRDYV

SEQ ID NO: 3 - protein, 220 aa, Homo sapiens
MSMGLEITGTALAVLGWLGTIVCCALPMWRVSAFIGSNIITSQNIWEGLWMNCVVQSTGQMQCKVYDSLLALPQDLQAARALIVVAILLAAFGLLVALVGAQCTNCVQDDTAKAKITIVAGVLFLLAALLTLVPVSWSANTIIRDFYNPVVPEAQKREMGAGLYVGWAAAALQLLGGALLCCSCPPREKKYTATKVVYSAPRSTGPGASLGTGYDRKDYV

SEQ ID NO: 4 - protein, 209 aa, Homo sapiens
MASMGLQVMGIALAVLGWLAVMLCCALPMWRVTAFIGSNIVTSQTIWEGLWMNCVVQSTGQMQCKVYDSLLALPQDLQAARALVIISIIVAALGVLLSVVGGKCTNCLEDESAKAKTMIVAGVVFLLAGLMVIVPVSWTAHNIIQDFYNPLVASGQKREMGASLYVGWAASGLLLLGGGLLCCNCPPRTDKPYSAKYSAARSAAASNYV

SEQ ID NO: 5 - protein, 219 aa, Mus musculus
MASTGLQILGIVLTLLGWVNALVSCALPMWKVTAFIGNSIVVAQMVWEGLWMSCVVQSTGQMQCKVYDSLLALPQDLQAARALCVVTLLIVLLGLLVYLAGAKCTTCVEDRNSKSRLVLISGIIFVISGVLTLIPVCWTAHSIIQDFYNPLVADAQKRELGASLYLGWAASGLLLLGGGLLCCACSSGGTQGPRHYMACYSTSVPHSRGPSEYPTKNYV

SEQ ID NO: 6 - protein, 41 aa, Artificial Sequence
  Peptide
LLCCTCPSGGSQGPSHYMARYSTSAPAISRGPSEYPTKNYV

SEQ ID NO: 7 - protein, 40 aa, Artificial Sequence
  Peptide
LLCCACSSGGTQGPRHYMACYSTSVPHSRGPSEYPTKNYV

SEQ ID NO: 8 - protein, 38 aa, Artificial Sequence
  Peptide
CTCPSGGSQGPSHYMARYSTSAPAISRGPSEYPTKNYV

SEQ ID NO: 9 - protein, 14 aa, Artificial Sequence
  Peptide
CTCPSGGSQGPSHY

SEQ ID NO: 10 - protein, 15 aa, Artificial Sequence
  Peptide
PSGGSQGPSHYMARY

SEQ ID NO: 11 - protein, 15 aa, Artificial Sequence
  Peptide
SQGPSHYMARYSTSA

SEQ ID NO: 12 - protein, 15 aa, Artificial Sequence
  Peptide
SHYMARYSTSAPAIS

SEQ ID NO: 13 - protein, 15 aa, Artificial Sequence
  Peptide
ARYSTSAPAISRGPS

SEQ ID NO: 14 - protein, 15 aa, Artificial Sequence
  Peptide
TSAPAISRGPSEYPT

SEQ ID NO: 15 - protein, 15 aa, Artificial Sequence
  Peptide
AISRGPSEYPTKNYV

SEQ ID NO: 16 - protein, 15 aa, Artificial Sequence
  Peptide
YMARYSTSAPAISRG

SEQ ID NO: 17 - protein, 15 aa, Artificial Sequence
  Peptide
RYSTSAPAISRGPSE

SEQ ID NO: 18 - protein, 15 aa, Artificial Sequence
  Peptide
YSTSAPAISRGPSEY

SEQ ID NO: 19 - protein, 15 aa, Artificial Sequence
  Peptide
STSAPAISRGPSEYP

SEQ ID NO: 20 - protein, 15 aa, Artificial Sequence
  Peptide
SAPAISRGPSEYPTK

SEQ ID NO: 21 - protein, 15 aa, Artificial Sequence
  Peptide
APAISRGPSEYPTKN

SEQ ID NO: 22 - protein, 15 aa, Artificial Sequence
  Peptide
PAISRGPSEYPTKNY

SEQ ID NO: 23 - protein, 14 aa, Artificial Sequence
  Peptide
ISRGPSEYPTKNYV

SEQ ID NO: 24 - protein, 13 aa, Artificial Sequence
  Peptide
SRGPSEYPTKNYV

SEQ ID NO: 25 - protein, 12 aa, Artificial Sequence
  Peptide
RGPSEYPTKNYV

SEQ ID NO: 26 - protein, 11 aa, Artificial Sequence
  Peptide
GPSEYPTKNYV

SEQ ID NO: 27 - protein, 10 aa, Artificial Sequence
  Peptide
PSEYPTKNYV

SEQ ID NO: 28 - protein, 9 aa, Artificial Sequence
  Peptide
SEYPTKNYV

SEQ ID NO: 29 - protein, 8 aa, Artificial Sequence
  Peptide
EYPTKNYV

SEQ ID NO: 30 - protein, 7 aa, Artificial Sequence
  Peptide
YPTKNYV

SEQ ID NO: 31 - protein, 6 aa, Artificial Sequence
  Peptide
PTKNYV

SEQ ID NO: 32 - protein, 5 aa, Artificial Sequence
  Peptide
PTKNY

SEQ ID NO: 33 - protein, 4 aa, Artificial Sequence
  Peptide
PTKN

SEQ ID NO: 34 - protein, 40 aa, Artificial Sequence
  Peptide
LCCTCPSGGSQGPSHYMARYSTSAPAISRGPSEYPTKNYV

SEQ ID NO: 35 - protein, 37 aa, Artificial Sequence
  Peptide
LCCTCPPPQVERPRGPRLGYSIPSRSGASGLDKRDYV

SEQ ID NO: 36 - protein, 41 aa, Artificial Sequence
  Peptide
LCCSCPPREKKYTATKVVYSAPRSTGPGASLGTGYDRKDYV

SEQ ID NO: 37 - protein, 29 aa, Artificial Sequence
  Peptide
LCCNCPPRTDKPYSAKYSAARSAAASNYV

SEQ ID NO: 38 - protein, 7 aa, Artificial Sequence
  Peptide
EYPTKNY

SEQ ID NO: 39 - protein, 4 aa, Artificial Sequence
  Peptide
RGPS

SEQ ID NO: 40 - protein, 114 aa, Artificial Sequence
  Antibody chain
EVQLQQSGTVLARPGASVRMSCRTSGYIFTTYWIHWVKERPGQGLVWIGAIFPGNSDTTYNQKFRGKASLTAVTSASTAYLDLSSLTDEDSAVYYCTREFYATWGQGTTLTVSS

SEQ ID NO: 41 - protein, 112 aa, Artificial Sequence
  Antibody chain
DIVLTQNPLTLSVTIGQTASISCKSSQNLLYSDGKTYLNWLLQRPGQSPKRLIYLMSKLDSGVPDRFTGSGSGTDFTLKISRVEAEDLGVYYCWQGTHFPWTFGGGTKLENT

SEQ ID NO: 42 - protein, 114 aa, Artificial Sequence
  Antibody chain
EVQLQQSGTVLARPGASVKMSCRTSGYTFTTYWMHWVRERPGQGLEWIGAIYPENSDATYNQKFKGKASLTAVTSASTAYLELSSLTDEDSAVYYCTREFYATWGQGTTLTVSS

SEQ ID NO: 43 - protein, 112 aa, Artificial Sequence
  Antibody chain
DVVMTQNPLTLSVTIGQTASISCKSSQNLLYSDGKTYLNWLLQRPGQSPKRLIYLMSKLDSGVPDRFTGSGSRTDFTLKISRVEAEDLGVYYCWQGTHFPWTFGGGTKLEIT

SEQ ID NO: 44 - protein, 114 aa, Artificial Sequence; identical to SEQ ID NO: 42
  Antibody chain

SEQ ID NO: 45 - protein, 112 aa, Artificial Sequence
  Antibody chain
DIVLTQNPLTLSVTIGQTASISCKSSQNLLYSDGKTYLNWLLQRPGQSPKRLIYLMSKLESGVPDRFTGSGSGTEFTLKISRVEAEDLGVYYCWQGTHFPWTFGGGTKLEIS

SEQ ID NO: 46 - protein, 17 aa, Artificial Sequence
  Peptide
CRDFYNPLVAEAQKREL

SEQ ID NO: 47 - protein, 20 aa, Artificial Sequence
  Peptide
GGGLLCCTCPSGGSQGPSHY

SEQ ID NO: 48 - protein, 21 aa, Artificial Sequence
  Peptide
CARYSTSAPAISRGPSEYPTK

SEQ ID NO: 49 - protein, 39 aa, Artificial Sequence
  Peptide
CCTCPSGGSQGPSHYMARYSTSAPAISRGPSEYPTKNYV

SEQ ID NO: 50 - protein, 61 aa, Artificial Sequence
  Peptide
AKCTTCVEEKDSKARLVLTSGIVFVISGVLTLIPVCWTAHAIIRDFYNPLVAEAQKRELGA

SEQ ID NO: 51 - protein, 8 aa, Artificial Sequence
  Variable heavy chain CDR
GYIFTTYW

SEQ ID NO: 52 - protein, 8 aa, Artificial Sequence
  Variable heavy chain CDR
IFPGNSDT

SEQ ID NO: 53 - protein, 7 aa, Artificial Sequence
  Variable heavy chain CDR
TREFYAT

SEQ ID NO: 54 - protein, 11 aa, Artificial Sequence
  Variable light chain CDR
QNLLYSDGKTY

SEQ ID NO: 55 - protein, 3 aa, Artificial Sequence
  Variable light chain CDR
LMS

SEQ ID NO: 56 - protein, 9 aa, Artificial Sequence
  Variable light chain CDR
WQGTHFPWT

SEQ ID NO: 57 - protein, 8 aa, Artificial Sequence
  Variable heavy chain CDR
GYTFTTYW

SEQ ID NO: 58 - protein, 8 aa, Artificial Sequence
  Variable heavy chain CDR
IYPENSDA

SEQ ID NO: 59 - protein, 5 aa, Artificial Sequence
  Peptide
EYPTK

SEQ ID NO: 60 - protein, 6 aa, Artificial Sequence
  Peptide
EYPTKN

SEQ ID NO: 61 - protein, 6 aa, Artificial Sequence
  Peptide
YPTKNY